European Patent Application EP 4 613 288 A1, published September 10, 2025. Title: FORMULATION OF AN ANTI-APC MONOCLONAL ANTIBODY AND USE THEREOF. Applicant: Oklahoma Medical Research Foundation. Application WO PCT/CN2023/108571, filed July 21, 2023. The sequence listing filed with the application follows.

SEQUENCE LISTING (6 sequences)

SEQ ID NO: 1 - protein, 218 aa, synthetic construct
DIQLTQSPSSLSASVGDRVTITCRASESVDSFGATFMHWYQQKPGKAPKLLIYLASRLGSGVPSRFSGSGSGTDFTLTISSLQPEDFATYYCQQNNEDPYTFGQGTKLEIKRTVAAPSVFIFPPSDEQLKSGTASVVCLLNNFYPREAKVQWKVDNALQSGNSQESVTEQDSKDSTYSLSSTLTLSKADYEKHKVYACEVTHQGLSSPVTKSFNRGEC

SEQ ID NO: 2 - protein, 445 aa, synthetic construct
EVQLVESGGGLVQPGGSLRLSCAASGFTFSFYYLNWVRQAPGKGLEWVGDIRLKKNNYEKHYAESVKGRFTISRDDSKSITYLQMNSLRAEDTAVYYCAREGDYFDYWGQGTTVTVSSASTKGPSVFPLAPCSRSTSESTAALGCLVKDYFPEPVTVSWNSGALTSGVHTFPAVLQSSGLYSLSSVVTVPSSSLGTKTYTCNVDHKPSNTKVDKRVESKYGPPCPPCPAPEFLGGPSVFLFPPKPKDTLMISRTPEVTCVVVDVSQEDPEVQFNWYVDGVEVHNAKTKPREEQFNSTYRVVSVLTVLHQDWLNGKEYKCKVSNKGLPSSIEKTISKAKGQPREPQVYTLPPSQEEMTKNQVSLTCLVKGFYPSDIAVEWESNGQPENNYKTTPPVLDSDGSFFLYSRLTVDKSRWQEGNVFSCSVMHEALHNHYTQKSLSLSLGK

SEQ ID NO: 3 - protein, 218 aa, synthetic construct; identical to SEQ ID NO: 1

SEQ ID NO: 4 - protein, 444 aa, synthetic construct
EVQLVESGGGLVQPGGSLRLSCAASGFTFSFYYLNWVRQAPGKGLEWVGDIRLKKNNYEKHYAESVKGRFTISRDDSKSITYLQMNSLRAEDTAVYYCAREGDYFDYWGQGTTVTVSSASTKGPSVFPLAPCSRSTSESTAALGCLVKDYFPEPVTVSWNSGALTSGVHTFPAVLQSSGLYSLSSVVTVPSSNFGTQTYTCNVDHKPSNTKVDKTVERKCCVECPPCPAPPVAGPSVFLFPPKPKDTLMISRTPEVTCVVVDVSHEDPEVQFNWYVDGVEVHNAKTKPREEQFNSTFRVVSVLTVVHQDWLNGKEYKCKVSNKGLPAPIEKTISKTKGQPREPQVYTLPPSREEMTKNQVSLTCLVKGFYPSDIAVEWESNGQPENNYKTTPPMLDSDGSFFLYSKLTVDKSRWQQGNVFSCSVMHEALHNHYTQKSLSLSPGK

SEQ ID NO: 5 - protein, 111 aa, synthetic construct
DIQLTQSPSSLSASVGDRVTITCRASESVDSFGATFMHWYQQKPGKAPKLLIYLASRLGSGVPSRFSGSGSGTDFTLTISSLQPEDFATYYCQQNNEDPYTFGQGTKLEIK

SEQ ID NO: 6 - protein, 118 aa, synthetic construct
EVQLVESGGGLVQPGGSLRLSCAASGFTFSFYYLNWVRQAPGKGLEWVGDIRLKKNNYEKHYAESVKGRFTISRDDSKSITYLQMNSLRAEDTAVYYCAREGDYFDYWGQGTTVTVSS